European Patent Specification EP 3 998 067 B1, published September 11, 2024. Title: COMPOSITIONS AND METHODS FOR TREATMENT OF HOMOCYSTINURIA. Applicant: The Regents of the University of Colorado, a body corporate. Application PCT/US2016/XXXXX. The sequence listing filed with the application follows.

SEQUENCE LISTING (16 sequences)

SEQ ID NO: 1 - DNA, 1656 bp, Homo sapiens
atgccgtcagaaaccccgcaggcagaagtgggtccgacgggttgcccgcaccgtagcggtccgcattctgcaaaaggcagtctggaaaaaggttccccggaagataaagaagccaaagaaccgctgtggattcgtccggacgcaccgtcacgctgtacctggcagctgggtcgtccggcaagcgaatctccgcatcaccatacggctccggcgaaaagtccgaaaattctgccggatatcctgaagaaaattggtgacaccccgatggttcgtatcaacaaaatcggcaaaaaattcggtctgaaatgcgaactgctggctaaatgtgaatttttcaatgcgggcggttccgtgaaagatcgtatctcactgcgcatgattgaagatgctgaacgcgacggcaccctgaaaccgggtgatacgattatcgaaccgacctctggcaacacgggtatcggtctggcactggcggcggcagtccgtggttatcgctgcattatcgtgatgccggaaaaaatgagctctgaaaaagttgatgtcctgcgtgctctgggcgcggaaattgttcgtaccccgacgaatgcccgcttcgacagtccggaatcccatgtgggtgttgcatggcgcctgaaaaacgaaatcccgaattcgcacattctggatcagtatcgtaacgctagcaatccgctggcgcattacgataccacggccgacgaaatcctgcagcaatgtgatggcaaactggacatgctggtcgcttctgtgggtaccggcggtaccattacgggcatcgcgcgtaaactgaaagaaaaatgcccgggctgtcgcattatcggtgtggatccggaaggcagtattctggcggaaccggaagaactgaaccagaccgaacaaaccacgtatgaagttgaaggcatcggttacgattttattccgaccgtcctggatcgcacggtggttgacaaatggttcaaaagcaatgacgaagaagcctttaccttcgcacgtatgctgatcgctcaggaaggtctgctgtgcggtggttcagcaggttcgacggtcgcagtggcagttaaagctgcgcaggaactgcaagaaggtcaacgttgtgtcgtgattctgccggattctgttcgcaactacatgaccaaatttctgagtgaccgttggatgctgcaaaaaggcttcctgaaagaagaagatctgaccgagaaaaaaccgtggtggtggcacctgcgcgtgcaggaactgggtctgtccgcaccgctgaccgttctgccgaccatcacgtgcggccatacgattgaaatcctgcgtgaaaaaggttttgatcaggccccggttgtcgacgaagcaggcgtgattctgggtatggttaccctgggtaacatgctgagttccctgctggcgggcaaagtgcaaccgagcgatcaggttggtaaagtcatctacaaacaattcaaacagattcgtctgaccgatacgctgggccgcctgtcgcacatcctggaaatggaccatttcgcgctggttgtgcacgaacagattcaataccatagcaccggcaaatcatcgcagcgccaaatggtctttggtgtcgtgacggccattgatctgctgaatttcgtggccgcacaagaacgtgaccagaaataa

SEQ ID NO: 2 - protein, 551 aa, Homo sapiens
MPSETPQAEVGPTGCPHRSGPHSAKGSLEKGSPEDKEAKEPLWIRPDAPSRCTWQLGRPASESPHHHTAPAKSPKILPDILKKIGDTPMVRINKIGKKFGLKCELLAKCEFFNAGGSVKDRISLRMIEDAERDGTLKPGDTIIEPTSGNTGIGLALAAAVRGYRCIIVMPEKMSSEKVDVLRALGAEIVRTPTNARFDSPESHVGVAWRLKNEIPNSHILDQYRNASNPLAHYDTTADEILQQCDGKLDMLVASVGTGGTITGIARKLKEKCPGCRIIGVDPEGSILAEPEELNQTEQTTYEVEGIGYDFIPTVLDRTVVDKWFKSNDEEAFTFARMLIAQEGLLCGGSAGSTVAVAVKAAQELQEGQRCVVILPDSVRNYMTKFLSDRWMLQKGFLKEEDLTEKKPWWWHLRVQELGLSAPLTVLPTITCGHTIEILREKGFDQAPVVDEAGVILGMVTLGNMLSSLLAGKVQPSDQVGKVIYKQFKQIRLTDTLGRLSHILEMDHFALVVHEQIQYHSTGKSSQRQMVFGVVTAIDLLNFVAAQERDQK

SEQ ID NO: 3 - protein, 413 aa, Artificial Sequence
  Synthetic
MPSETPQAEVGPTGCPHRSGPHSAKGSLEKGSPEDKEAKEPLWIRPDAPSRCTWQLGRPASESPHHHTAPAKSPKILPDILKKIGDTPMVRINKIGKKFGLKCELLAKCEFFNAGGSVKDRISLRMIEDAERDGTLKPGDTIIEPTSGNTGIGLALAAAVRGYRCIIVMPEKMSSEKVDVLRALGAEIVRTPTNARFDSPESHVGVAWRLKNEIPNSHILDQYRNASNPLAHYDTTADEILQQCDGKLDMLVASVGTGGTITGIARKLKEKCPGCRIIGVDPEGSILAEPEELNQTEQTTYEVEGIGYDFIPTVLDRTVVDKWFKSNDEEAFTFARMLIAQEGLLCGGSAGSTVAVAVKAAQELQEGQRCVVILPDSVRNYMTKFLSDRWMLQKGFLKEEDLTEKKPWWWHLR

SEQ ID NO: 4 - DNA, 1242 bp, Artificial Sequence
  Synthetic
atgccgtcagaaaccccgcaggcagaagtgggtccgacgggttgcccgcaccgtagcggtccgcattctgcaaaaggcagtctggaaaaaggttccccggaagataaagaagccaaagaaccgctgtggattcgtccggacgcaccgtcacgctgtacctggcagctgggtcgtccggcaagcgaatctccgcatcaccatacggctccggcgaaaagtccgaaaattctgccggatatcctgaagaaaattggtgacaccccgatggttcgtatcaacaaaatcggcaaaaaattcggtctgaaatgcgaactgctggctaaatgtgaatttttcaatgcgggcggttccgtgaaagatcgtatctcactgcgcatgattgaagatgctgaacgcgacggcaccctgaaaccgggtgatacgattatcgaaccgacctctggcaacacgggtatcggtctggcactggcggcggcagtccgtggttatcgctgcattatcgtgatgccggaaaaaatgagctctgaaaaagttgatgtcctgcgtgctctgggcgcggaaattgttcgtaccccgacgaatgcccgcttcgacagtccggaatcccatgtgggtgttgcatggcgcctgaaaaacgaaatcccgaattcgcacattctggatcagtatcgtaacgctagcaatccgctggcgcattacgataccacggccgacgaaatcctgcagcaatgtgatggcaaactggacatgctggtcgcttctgtgggtaccggcggtaccattacgggcatcgcgcgtaaactgaaagaaaaatgcccgggctgtcgcattatcggtgtggatccggaaggcagtattctggcggaaccggaagaactgaaccagaccgaacaaaccacgtatgaagttgaaggcatcggttacgattttattccgaccgtcctggatcgcacggtggttgacaaatggttcaaaagcaatgacgaagaagcctttaccttcgcacgtatgctgatcgctcaggaaggtctgctgtgcggtggttcagcaggttcgacggtcgcagtggcagttaaagctgcgcaggaactgcaagaaggtcaacgttgtgtcgtgattctgccggattctgttcgcaactacatgaccaaatttctgagtgaccgttggatgctgcaaaaaggcttcctgaaagaagaagatctgaccgagaaaaaaccgtggtggtggcacctgcgctaa

SEQ ID NO: 5 - DNA, 30 bp, Artificial Sequence
  Synthetic oligonucleotide
cgtagaattcacctttgcccgcatgctgat

SEQ ID NO: 6 - DNA, 35 bp, Artificial Sequence
  Synthetic oligonucleotide
tacgggtacctcaacggaggtgccaccaccagggc

SEQ ID NO: 7 - DNA, 29 bp, Artificial Sequence
  Synthetic oligonucleotide
agtcgcccatggcgtcagaaaccccgcag

SEQ ID NO: 8 - DNA, 31 bp, Artificial Sequence
  Synthetic oligonucleotide
atcgcgctcgagttagcgcaggtgccaccac

SEQ ID NO: 9 - DNA, 30 bp, Artificial Sequence
  Synthetic oligonucleotide
ggagatataccatgccgtcagaaaccccgc

SEQ ID NO: 10 - DNA, 30 bp, Artificial Sequence
  Synthetic oligonucleotide
gcggggtttctgacggcatggtatatctcc

SEQ ID NO: 11 - DNA, 23 bp, Artificial Sequence
  Synthetic oligonucleotide
tgggtccgacgggtagcccgcac

SEQ ID NO: 12 - DNA, 23 bp, Artificial Sequence
  Synthetic oligonucleotide
gtgcgggctacccgtcggaccca

SEQ ID NO: 13 - protein, 413 aa, Artificial Sequence
  Truncated human C15S mutant CBS polypeptide
MPSETPQAEVGPTGSPHRSGPHSAKGSLEKGSPEDKEAKEPLWIRPDAPSRCTWQLGRPASESPHHHTAPAKSPKILPDILKKIGDTPMVRINKIGKKFGLKCELLAKCEFFNAGGSVKDRISLRMIEDAERDGTLKPGDTIIEPTSGNTGIGLALAAAVRGYRCIIVMPEKMSSEKVDVLRALGAEIVRTPTNARFDSPESHVGVAWRLKNEIPNSHILDQYRNASNPLAHYDTTADEILQQCDGKLDMLVASVGTGGTITGIARKLKEKCPGCRIIGVDPEGSILAEPEELNQTEQTTYEVEGIGYDFIPTVLDRTVVDKWFKSNDEEAFTFARMLIAQEGLLCGGSAGSTVAVAVKAAQELQEGQRCVVILPDSVRNYMTKFLSDRWMLQKGFLKEEDLTEKKPWWWHLR

SEQ ID NO: 14 - DNA, 1242 bp, Artificial Sequence
  Truncated human C15S mutant CBS Nucleotide
atgccgtcagaaaccccgcaggcagaagtgggtccgacgggtagcccgcaccgtagcggtccgcattctgcaaaaggcagtctggaaaaaggttccccggaagataaagaagccaaagaaccgctgtggattcgtccggacgcaccgtcacgctgtacctggcagctgggtcgtccggcaagcgaatctccgcatcaccatacggctccggcgaaaagtccgaaaattctgccggatatcctgaagaaaattggtgacaccccgatggttcgtatcaacaaaatcggcaaaaaattcggtctgaaatgcgaactgctggctaaatgtgaatttttcaatgcgggcggttccgtgaaagatcgtatctcactgcgcatgattgaagatgctgaacgcgacggcaccctgaaaccgggtgatacgattatcgaaccgacctctggcaacacgggtatcggtctggcactggcggcggcagtccgtggttatcgctgcattatcgtgatgccggaaaaaatgagctctgaaaaagttgatgtcctgcgtgctctgggcgcggaaattgttcgtaccccgacgaatgcccgcttcgacagtccggaatcccatgtgggtgttgcatggcgcctgaaaaacgaaatcccgaattcgcacattctggatcagtatcgtaacgctagcaatccgctggcgcattacgataccacggccgacgaaatcctgcagcaatgtgatggcaaactggacatgctggtcgcttctgtgggtaccggcggtaccattacgggcatcgcgcgtaaactgaaagaaaaatgcccgggctgtcgcattatcggtgtggatccggaaggcagtattctggcggaaccggaagaactgaaccagaccgaacaaaccacgtatgaagttgaaggcatcggttacgattttattccgaccgtcctggatcgcacggtggttgacaaatggttcaaaagcaatgacgaagaagcctttaccttcgcacgtatgctgatcgctcaggaaggtctgctgtgcggtggttcagcaggttcgacggtcgcagtggcagttaaagctgcgcaggaactgcaagaaggtcaacgttgtgtcgtgattctgccggattctgttcgcaactacatgaccaaatttctgagtgaccgttggatgctgcaaaaaggcttcctgaaagaagaagatctgaccgagaaaaaaccgtggtggtggcacctgcgctaa

SEQ ID NO: 15 - DNA, 1656 bp, Artificial Sequence
  Full length human C15S mutant CBS nucleotide
atgccgtcagaaaccccgcaggcagaagtgggtccgacgggtagcccgcaccgtagcggtccgcattctgcaaaaggcagtctggaaaaaggttccccggaagataaagaagccaaagaaccgctgtggattcgtccggacgcaccgtcacgctgtacctggcagctgggtcgtccggcaagcgaatctccgcatcaccatacggctccggcgaaaagtccgaaaattctgccggatatcctgaagaaaattggtgacaccccgatggttcgtatcaacaaaatcggcaaaaaattcggtctgaaatgcgaactgctggctaaatgtgaatttttcaatgcgggcggttccgtgaaagatcgtatctcactgcgcatgattgaagatgctgaacgcgacggcaccctgaaaccgggtgatacgattatcgaaccgacctctggcaacacgggtatcggtctggcactggcggcggcagtccgtggttatcgctgcattatcgtgatgccggaaaaaatgagctctgaaaaagttgatgtcctgcgtgctctgggcgcggaaattgttcgtaccccgacgaatgcccgcttcgacagtccggaatcccatgtgggtgttgcatggcgcctgaaaaacgaaatcccgaattcgcacattctggatcagtatcgtaacgctagcaatccgctggcgcattacgataccacggccgacgaaatcctgcagcaatgtgatggcaaactggacatgctggtcgcttctgtgggtaccggcggtaccattacgggcatcgcgcgtaaactgaaagaaaaatgcccgggctgtcgcattatcggtgtggatccggaaggcagtattctggcggaaccggaagaactgaaccagaccgaacaaaccacgtatgaagttgaaggcatcggttacgattttattccgaccgtcctggatcgcacggtggttgacaaatggttcaaaagcaatgacgaagaagcctttaccttcgcacgtatgctgatcgctcaggaaggtctgctgtgcggtggttcagcaggttcgacggtcgcagtggcagttaaagctgcgcaggaactgcaagaaggtcaacgttgtgtcgtgattctgccggattctgttcgcaactacatgaccaaatttctgagtgaccgttggatgctgcaaaaaggcttcctgaaagaagaagatctgaccgagaaaaaaccgtggtggtggcacctgcgcgtgcaggaactgggtctgtccgcaccgctgaccgttctgccgaccatcacgtgcggccatacgattgaaatcctgcgtgaaaaaggttttgatcaggccccggttgtcgacgaagcaggcgtgattctgggtatggttaccctgggtaacatgctgagttccctgctggcgggcaaagtgcaaccgagcgatcaggttggtaaagtcatctacaaacaattcaaacagattcgtctgaccgatacgctgggccgcctgtcgcacatcctggaaatggaccatttcgcgctggttgtgcacgaacagattcaataccatagcaccggcaaatcatcgcagcgccaaatggtctttggtgtcgtgacggccattgatctgctgaatttcgtggccgcacaagaacgtgaccagaaataa

SEQ ID NO: 16 - protein, 551 aa, Artificial Sequence
  Full length human C15S mutant CBS polypeptide
MPSETPQAEVGPTGSPHRSGPHSAKGSLEKGSPEDKEAKEPLWIRPDAPSRCTWQLGRPASESPHHHTAPAKSPKILPDILKKIGDTPMVRINKIGKKFGLKCELLAKCEFFNAGGSVKDRISLRMIEDAERDGTLKPGDTIIEPTSGNTGIGLALAAAVRGYRCIIVMPEKMSSEKVDVLRALGAEIVRTPTNARFDSPESHVGVAWRLKNEIPNSHILDQYRNASNPLAHYDTTADEILQQCDGKLDMLVASVGTGGTITGIARKLKEKCPGCRIIGVDPEGSILAEPEELNQTEQTTYEVEGIGYDFIPTVLDRTVVDKWFKSNDEEAFTFARMLIAQEGLLCGGSAGSTVAVAVKAAQELQEGQRCVVILPDSVRNYMTKFLSDRWMLQKGFLKEEDLTEKKPWWWHLRVQELGLSAPLTVLPTITCGHTIEILREKGFDQAPVVDEAGVILGMVTLGNMLSSLLAGKVQPSDQVGKVIYKQFKQIRLTDTLGRLSHILEMDHFALVVHEQIQYHSTGKSSQRQMVFGVVTAIDLLNFVAAQERDQK